European Patent Application EP 4 733 298 A1, published April 29, 2026. Title: NOVEL TRPM4 ANTAGONISTS AND MEDICAL USE THEREOF. Applicant: Universitätsklinikum Hamburg-Eppendorf. Application EP. The sequence listing filed with the application follows.

SEQUENCE LISTING (17 sequences)

SEQ ID NO: 1 - protein, 1214 aa, Homo sapiens
MVVPEKEQSWIPKIFKKKTCTTFIVDSTDPGGTLCQCGRPRTAHPAVAMEDAFGAAVVTVWDSDAHTTEKPTDAYGELDFTGAGRKHSNFLRLSDRTDPAAVYSLVTRTWGFRAPNLVVSVLGGSGGPVLQTWLQDLLRRGLVRAAQSTGAWIVTGGLHTGIGRHVGVAVRDHQMASTGGTKVVAMGVAPWGVVRNRDTLINPKGSFPARYRWRGDPEDGVQFPLDYNYSAFFLVDDGTHGCLGGENRFRLRLESYISQQKTGVGGTGIDIPVLLLLIDGDEKMLTRIENATQAQLPCLLVAGSGGAADCLAETLEDTLAPGSGGARQGEARDRIRRFFPKGDLEVLQAQVERIMTRKELLTVYSSEDGSEEFETIVLKALVKACGSSEASAYLDELRLAVAWNRVDIAQSELFRGDIQWRSFHLEASLMDALLNDRPEFVRLLISHGLSLGHFLTPMRLAQLYSAAPSNSLIRNLLDQASHSAGTKAPALKGGAAELRPPDVGHVLRMLLGKMCAPRYPSGGAWDPHPGQGFGESMYLLSDKATSPLSLDAGLGQAPWSDLLLWALLLNRAQMAMYFWEMGSNAVSSALGACLLLRVMARLEPDAEEAARRKDLAFKFEGMGVDLFGECYRSSEVRAARLLLRRCPLWGDATCLQLAMQADARAFFAQDGVQSLLTQKWWGDMASTTPIWALVLAFFCPPLIYTRLITFRKSEEEPTREELEFDMDSVINGEGPVGTADPAEKTPLGVPRQSGRPGCCGGRCGGRRCLRRWFHFWGAPVTIFMGNVVSYLLFLLLFSRVLLVDFQPAPPGSLELLLYFWAFTLLCEELRQGLSGGGGSLASGGPGPGHASLSQRLRLYLADSWNQCDLVALTCFLLGVGCRLTPGLYHLGRTVLCIDFMVFTVRLLHIFTVNKQLGPKIVIVSKMMKDVFFFLFFLGVWLVAYGVATEGLLRPRDSDFPSILRRVFYRPYLQIFGQIPQEDMDVALMEHSNCSSEPGFWAHPPGAQAGTCVSQYANWLVVLLLVIFLLVANILLVNLLIAMFSYTFGKVQGNSDLYWKAQRYRLIREFHSRPALAPPFIVISHLRLLLRQLCRRPRSPQPSSPALEHFRVYLSKEAERKLLTWESVHKENFLLARARDKRESDSERLKRTSQKVDLALKQLGHIREYEQRLKVLEREVQQCSRVLGWVAEALSRSALLPPGGPPPPDLPGSKD

SEQ ID NO: 2 - protein, 1069 aa, Homo sapiens
MVVPEKEQSWIPKIFKKKTCTTFIVDSTDPGGTLCQCGRPRTAHPAVAMEDAFGAAVVTVWDSDAHTTEKPTDAYGELDFTGAGRKHSNFLRLSDRTDPAAVYSLVTRTWGFRAPNLVVSVLGGSGGPVLQTWLQDLLRRGLVRAAQSTGAWIVTGGLHTGIGRHVGVAVRDHQMASTGGTKVVAMGVAPWGVVRNRDTLINPKGSFPARYRWRGDPEDGVQFPLDYNYSAFFLVDDGTHGCLGGENRFRLRLESYISQQKTGVGGTGIDIPVLLLLIDGDEKMLTRIENATQAQLPCLLVAGSGGAADCLAETLEDTLAPGSGGARQGEARDRIRRFFPKGDLEVLQAQVERIMTRKELLTVYSSEDGSEEFETIVLKALVKACGSSEASAYLDELRLAVAWNRVDIAQSELFRGDIQWRSFHLEASLMDALLNDRPEFVRLLISHGLSLGHFLTPMRLAQLYSAAPSNSLIRNLLDQASHSAGTKAPALKGGAAELRPPDVGHVLRMLLGKMCAPRYPSGGAWDPHPGQGFGESMYLLSDKATSPLSLDAGLGQAPWSDLLLWALLLNRAQMAMYFWEMGSNAVSSALGACLLLRVMARLEPDAEEAARRKDLAFKFEGMGVDLFGECYRSSEVRAARLLLRRCPLWGDATCLQLAMQADARAFFAQDGVQSLLTQKWWGDMASTTPIWALVLAFFCPPLIYTRLITFRKSEEEPTREELEFDMDSVINGEGPVGLTPGLYHLGRTVLCIDFMVFTVRLLHIFTVNKQLGPKIVIVSKMMKDVFFFLFFLGVWLVAYGVATEGLLRPRDSDFPSILRRVFYRPYLQIFGQIPQEDMDVALMEHSNCSSEPGFWAHPPGAQAGTCVSQYANWLVVLLLVIFLLVANILLVNLLIAMFSYTFGKVQGNSDLYWKAQRYRLIREFHSRPALAPPFIVISHLRLLLRQLCRRPRSPQPSSPALEHFRVYLSKEAERKLLTWESVHKENFLLARARDKRESDSERLKRTSQKVDLALKQLGHIREYEQRLKVLEREVQQCSRVLGWVAEALSRSALLPPGGPPPPDLPGSKD

SEQ ID NO: 3 - protein, 1040 aa, Homo sapiens
MASTGGTKVVAMGVAPWGVVRNRDTLINPKGSFPARYRWRGDPEDGVQFPLDYNYSAFFLVDDGTHGCLGGENRFRLRLESYISQQKTGVGGTGIDIPVLLLLIDGDEKMLTRIENATQAQLPCLLVAGSGGAADCLAETLEDTLAPGSGGARQGEARDRIRRFFPKGDLEVLQAQVERIMTRKELLTVYSSEDGSEEFETIVLKALVKACGSSEASAYLDELRLAVAWNRVDIAQSELFRGDIQWRSFHLEASLMDALLNDRPEFVRLLISHGLSLGHFLTPMRLAQLYSAAPSNSLIRNLLDQASHSAGTKAPALKGGAAELRPPDVGHVLRMLLGKMCAPRYPSGGAWDPHPGQGFGESMYLLSDKATSPLSLDAGLGQAPWSDLLLWALLLNRAQMAMYFWEMGSNAVSSALGACLLLRVMARLEPDAEEAARRKDLAFKFEGMGVDLFGECYRSSEVRAARLLLRRCPLWGDATCLQLAMQADARAFFAQDGVQSLLTQKWWGDMASTTPIWALVLAFFCPPLIYTRLITFRKSEEEPTREELEFDMDSVINGEGPVGTADPAEKTPLGVPRQSGRPGCCGGRCGGRRCLRRWFHFWGAPVTIFMGNVVSYLLFLLLFSRVLLVDFQPAPPGSLELLLYFWAFTLLCEELRQGLSGGGGSLASGGPGPGHASLSQRLRLYLADSWNQCDLVALTCFLLGVGCRLTPGLYHLGRTVLCIDFMVFTVRLLHIFTVNKQLGPKIVIVSKMMKDVFFFLFFLGVWLVAYGVATEGLLRPRDSDFPSILRRVFYRPYLQIFGQIPQEDMDVALMEHSNCSSEPGFWAHPPGAQAGTCVSQYANWLVVLLLVIFLLVANILLVNLLIAMFSYTFGKVQGNSDLYWKAQRYRLIREFHSRPALAPPFIVISHLRLLLRQLCRRPRSPQPSSPALEHFRVYLSKEAERKLLTWESVHKENFLLARARDKRESDSERLKRTSQKVDLALKQLGHIREYEQRLKVLEREVQQCSRVLGWVAEALSRSALLPPGGPPPPDLPGSKD

SEQ ID NO: 4 - protein, 1165 aa, Homo sapiens
MQDVQGPRPGSPGDAEDRRELGLHRGEVNFGGSGKKRGKFVRVPSGVAPSVLFDLLLAEWHLPAPNLVVSLVGEEQPFAMKSWLRDVLRKGLVKAAQSTGAWILTSALRVGLARHVGQAVRDHSLASTSTKVRVVAVGMASLGRVLHRRILEEAQEDFPVHYPEDDGGSQGPLCSLDSNLSHFILVEPGPPGKGDGLTELRLRLEKHISEQRAGYGGTGSIEIPVLCLLVNGDPNTLERISRAVEQAAPWLILVGSGGIADVLAALVNQPHLLVPKVAEKQFKEKFPSKHFSWEDIVRWTKLLQNITSHQHLLTVYDFEQEGSEELDTVILKALVKACKSHSQEPQDYLDELKLAVAWDRVDIAKSEIFNGDVEWKSCDLEEVMVDALVSNKPEFVRLFVDNGADVADFLTYGRLQELYRSVSRKSLLFDLLQRKQEEARLTLAGLGTQQAREPPAGPPAFSLHEVSRVLKDFLQDACRGFYQDGRPGDRRRAEKGPAKRPTGQKWLLDLNQKSENPWRDLFLWAVLQNRHEMATYFWAMGQEGVAAALAACKILKEMSHLETEAEAARATREAKYERLALDLFSECYSNSEARAFALLVRRNRCWSKTTCLHLATEADAKAFFAHDGVQAFLTRIWWGDMAAGTPILRLLGAFLCPALVYTNLITFSEEAPLRTGLEDLQDLDSLDTEKSPLYGLQSRVEELVEAPRAQGDRGPRAVFLLTRWRKFWGAPVTVFLGNVVMYFAFLFLFTYVLLVDFRPPPQGPSGPEVTLYFWVFTLVLEEIRQGFFTDEDTHLVKKFTLYVGDNWNKCDMVAIFLFIVGVTCRMLPSAFEAGRTVLAMDFMVFTLRLIHIFAIHKQLGPKIIVVERMMKDVFFFLFFLSVWLVAYGVTTQALLHPHDGRLEWIFRRVLYRPYLQIFGQIPLDEIDEARVNCSTHPLLLEDSPSCPSLYANWLVILLLVTFLLVTNVLLMNLLIAMFSYTFQVVQGNADMFWKFQRYNLIVEYHERPALAPPFILLSHLSLTLRRVFKKEAEHKREHLERDLPDPLDQKVVTWETVQKENFLSKMEKRRRDSEGEVLRKTAHRVDFIAKYLGGLREQEKRIKCLESQINYCSVLVSSVADVLAQGGGPRSSQHCGEGSQLVAADHRGGLDGWEQPGAGQPPSDT

SEQ ID NO: 5 - protein, 1165 aa, Danio rerio
MVEKSSERFDKQMAGRLGDIDFTGVSRTRGKFVRVTSSTDPAEIYQILTKQWGLAPPHLVVALMGGDEVAQLKPWLRDTLRKGLVKAAQSTGAWILTSGLRFGITKNLGQAVRDHSLASTSPKVRVVAIGIAPWNMIQNRDLLLSAKPDHPATYPTEDLPYGAVYSLDCNHSHFILVDEDPKRPGATGEMRVKMLKHISLQRTGYGGTGSIEIPVLCLLVHGEPRILQKMYKNIQNSIPWLILAGSGGVADILVTLMDRGCWDADIVQELLINTFPDGLHSTEITSWTKLIQRILDHGHLLTVHDPEQDSELDTVILKALVKACKSQSQEAQDFLDELKLAVAWNRVDIAKSEIFSGDVQWSAQDLEEVMMEALVNDKPDFVRLFVDNGVNIKQFLTYGRLQELYCSVSEKNLLHTLLLKKNQERQAQLARKRMSGNPNNELGDRKFRFTFHEVSKVLKDFLDDTCKGFYQKLPAERMGKGRLFHSQKNLPDMDRRCEHPWRDLFLWAILQNRQEMANYFWAMGPEAVAAALVGCKIMKEMAHLATEAESARSMKNAKYEQFAMDLFSECYSNSEDRAYSLLVRKTCCWSKATVLNIATLAEAKCFFAHDGVQALLTKVWWGAMRTDTSISRLVLTFFIPPLVWTSLIKFNPEEQVSKDEGEPFAELDSLETEQALLLTDGDPVAGEGSAETAARSCSATFIRVVLRRWNRFWSAPVTVFMGNVIMYFAFLILFSYVLLLDFRPPPPYGPSAAEIILYFWVFTLVLEEIRQSFFTDEDMSILKKMKLYVEDNWNKCDMVAISLFVVGLSCRMAMSTYEAGRTVLALDFMVFTLRLIHIFAIHKQLGPKIIIVERMIKDVFFFLFFLSVWLIAYGVTTQALLHPNDPRIDWVFRRALYRPYLHIFGQIPLEEIDAAKMPDDNCTTDVQEIILGTLPPCPNIYANWLVILLLVIYLLVTNVLLLNLLIAMFSYTFQVVQENADIFWKFQRYNLIVEYHSRPALAPPFIIISHITQALLSFIKKTENTQDLLERELPSGLDQKLMTWETVQKENYLAKLEHEHRESSGERLRYTSSKVQTLLRMVGGFKDQEKRMATVETEVRYCGEVLSWIAECFHKSTLKCDRDAPKAPRSIAGSSRDQQPQGAKRQQPAGHPAYGTDKKLPFIDH

SEQ ID NO: 6 - protein, 1214 aa, synthetic construct
MVVPEKEQSWIPKIFKKKTCTTFIVDSTDPGGTLCQCGRPRTAHPAVAMEDAFGAAVVTVWDSDAHTTEKPTDAYGELDFTGAGRKHSNFLRLSDRTDPAAVYSLVTRTWGFRAPNLVVSVLGGSGGPVLQTWLQDLLRRGLVRAAQSTGAWIVTGGLHTGIGRHVGVAVRDHQMASTGGTKVVAMGVAPWGVVRNRDTLINPKGSFPARYRWRGDPEDGVQFPLDYNYSAFFLVDDGTHGCLGGENRFRLRLESYISQQKTGVGGTGIDIPVLLLLIDGDEKMLTRIENATQAQLPCLLVAGSGGAADCLAETLEDTLAPGSGGARQGEARDRIRRFFPKGDLEVLQAQVERIMTRKELLTVYSSEDGSEEFETIVLKALVKACGSSEASAYLDELRLAVAWNRVDIAQSELFRGDIQWRSFHLEASLMDALLNDRPEFVRLLISHGLSLGHFLTPMRLAQLYSAAPSNSLIRNLLDQASHSAGTKAPALKGGAAELRPPDVGHVLRMLLGKMCAPRYPSGGAWDPHPGQGFGESMYLLSDKATSPLSLDAGLGQAPWSDLLLWALLLNRAQMAMYFWEMGSNAVSSALGACLLLRVMARLEPDAEEAARRKDLAFKFEGMGVDLFGECYRSSEVRAARLLLRRCPLWGDATCLQLAMQADARAFFAQDGVQSLLTQKWWGDMASTTPIWALVLAFFCPPLIYTRLITFRKSEEEPTREELEFDMDSVINGEGPVGTADPAEKTPLGVPRQSGRPGCCGGRCGGRRCLRRWFHFWGAPVTIFMGNVVSYLLFLLLFSRVLLVDFQPAPPGSLELLLYFWAFTLLCEELRQGLSGGGGSLASGGPGPGHASLSQRLRLYLADSWNQCDLVALTCFLLGVGCRLTPGLYHLGRTVLCIDFMVFTVRLAHIFTVNKQLGPKIVIVSKMMKDVFFFLFFLGVWLVAYGVATEGLLRPRDSDFPSILRRVFYRPYLQIFGQIPQEDMDVALMEHSNCSSEPGFWAHPPGAQAGTCVSQYANWLVVLLLVIFLLVANILLVNLLIAMFSYTFGKVQGNSDLYWKAQRYRLIREFHSRPALAPPFIVISHLRLLLRQLCRRPRSPQPSSPALEHFRVYLSKEAERKLLTWESVHKENFLLARARDKRESDSERLKRTSQKVDLALKQLGHIREYEQRLKVLEREVQQCSRVLGWVAEALSRSALLPPGGPPPPDLPGSKD

SEQ ID NO: 7 - protein, 1214 aa, synthetic construct
MVVPEKEQSWIPKIFKKKTCTTFIVDSTDPGGTLCQCGRPRTAHPAVAMEDAFGAAVVTVWDSDAHTTEKPTDAYGELDFTGAGRKHSNFLRLSDRTDPAAVYSLVTRTWGFRAPNLVVSVLGGSGGPVLQTWLQDLLRRGLVRAAQSTGAWIVTGGLHTGIGRHVGVAVRDHQMASTGGTKVVAMGVAPWGVVRNRDTLINPKGSFPARYRWRGDPEDGVQFPLDYNYSAFFLVDDGTHGCLGGENRFRLRLESYISQQKTGVGGTGIDIPVLLLLIDGDEKMLTRIENATQAQLPCLLVAGSGGAADCLAETLEDTLAPGSGGARQGEARDRIRRFFPKGDLEVLQAQVERIMTRKELLTVYSSEDGSEEFETIVLKALVKACGSSEASAYLDELRLAVAWNRVDIAQSELFRGDIQWRSFHLEASLMDALLNDRPEFVRLLISHGLSLGHFLTPMRLAQLYSAAPSNSLIRNLLDQASHSAGTKAPALKGGAAELRPPDVGHVLRMLLGKMCAPRYPSGGAWDPHPGQGFGESMYLLSDKATSPLSLDAGLGQAPWSDLLLWALLLNRAQMAMYFWEMGSNAVSSALGACLLLRVMARLEPDAEEAARRKDLAFKFEGMGVDLFGECYRSSEVRAARLLLRRCPLWGDATCLQLAMQADARAFFAQDGVQSLLTQKWWGDMASTTPIWALVLAFFCPPLIYTRLITFRKSEEEPTREELEFDMDSVINGEGPVGTADPAEKTPLGVPRQSGRPGCCGGRCGGRRCLRRWFHFWGAPVTIFMGNVVSYLLFLLLFSRVLLVDFQPAPPGSLELLLYFWAFTLLCEELRQGLSGGGGSLASGGPGPGHASLSQRLRLYLADSWNQCDLVALTCFLLGVGCRLTPGLYHLGRTVLCIDFMVFTVRLLHIFTVNKQLGPKIVIVAKMMKDVFFFLFFLGVWLVAYGVATEGLLRPRDSDFPSILRRVFYRPYLQIFGQIPQEDMDVALMEHSNCSSEPGFWAHPPGAQAGTCVSQYANWLVVLLLVIFLLVANILLVNLLIAMFSYTFGKVQGNSDLYWKAQRYRLIREFHSRPALAPPFIVISHLRLLLRQLCRRPRSPQPSSPALEHFRVYLSKEAERKLLTWESVHKENFLLARARDKRESDSERLKRTSQKVDLALKQLGHIREYEQRLKVLEREVQQCSRVLGWVAEALSRSALLPPGGPPPPDLPGSKD

SEQ ID NO: 8 - protein, 1213 aa, Mus musculus
MVGPEKEQSWIPKIFRKKVCTTFIVDLSDDAGGTLCQCGQPRDAHPSVAVEDAFGAAVVTEWNSDEHTTEKPTDAYGDLDFTYSGRKHSNFLRLSDRTDPATVYSLVTRSWGFRAPNLVVSVLGGSGGPVLQTWLQDLLRRGLVRAAQSTGAWIVTGGLHTGIGRHVGVAVRDHQTASTGSSKVVAMGVAPWGVVRNRDMLINPKGSFPARYRWRGDPEDGVEFPLDYNYSAFFLVDDGTYGRLGGENRFRLRFESYVAQQKTGVGGTGIDIPVLLLLIDGDEKMLKRIEDATQAQLPCLLVAGSGGAADCLVETLEDTLAPGSGGLRRGEARDRIRRYFPKGDPEVLQAQVERIMTRKELLTVYSSEDGSEEFETIVLRALVKACGSSEASAYLDELRLAVAWNRVDIAQSELFRGDIQWRSFHLEASLMDALLNDRPEFVRLLISHGLSLGHFLTPVRLAQLYSAVSPNSLIRNLLDQASHASSSKSPPVNGTVELRPPNVGQVLRTLLGETCAPRYPARNTRDSYLGQDHRENDSLLMDWANKQPSTDASFEQAPWSDLLIWALLLNRAQMAIYFWEKGSNSVASALGACLLLRVMARLESEAEEAARRKDLAATFESMSVDLFGECYHNSEERAARLLLRRCPLWGEATCLQLAMQADARAFFAQDGVQSLLTQKWWGEMDSTTPIWALLLAFFCPPLIYTNLIVFRKSEEEPTQKDLDFDMDSSINGAGPPGTVEPSAKVALERRQRRRPGRALCCGKFSKRWSDFWGAPVTAFLGNVVSYLLFLLLFAHVLLVDFQPTKPSVSELLLYFWAFTLLCEELRQGLGGGWGSLASGGRGPDRAPLRHRLHLYLSDTWNQCDLLALTCFLLGVGCRLTPGLFDLGRTVLCLDFMIFTLRLLHIFTVNKQLGPKIVIVSKMMKDVFFFLFFLCVWLVAYGVATEGILRPQDRSLPSILRRVFYRPYLQIFGQIPQEEMDVALMIPGNCSMERGSWAHPEGPVAGSCVSQYANWLVVLLLIVFLLVANILLLNLLIAMFSYTFSKVHGNSDLYWKAQRYSLIREFHSRPALAPPLIIISHVRLLIKWLRRCRRCRRANLPASPVFEHFRVCLSKEAERKLLTWESVHKENFLLAQARDKRDSDSERLKRTSQKVDTALKQLGQIREYDRRLRGLEREVQHCSRVLTWMAEALSHSALLPPGAPPPPSPTGSKD

SEQ ID NO: 9 - protein, 1115 aa, Ficedula albicollis
MLDSSNLLLAFAVVYCSSISSSTTLFQVSMGSMRHRRNGNFESSRLLYSSMSRSIDVACSDADLANFIQENFKKRECVFFTKDTKSMGNLCKCGYPENQHIEGTQVNTTEKWNYKKHTKELPTDAFGDIQFENLGKRGKYIRLSCDTDSETLYDLMTQHWHLKTPNLVISVTGGAKNFALKPRMRKIFSRLIYIAQSKGAWIFTGGTHYGLMKYIGEVVRDNTISRSSEENVVAIGIAAWGMISNRETLIRTADSDGSYLAHYIMDDLKRDPLYCLDNNHTHLLLVDNGTHGHPTIEAKVRTQLEKYISERVIPESNYGGKIPIVCFAQGGGKETLKSINVAIKSKIPCVVVEGSGRIADVIASLVEAEGTLASSCVKESLLRFLPRTISRLSEEETESWIKWIKEVLESPHLLTVIKIEEAGDEIVSNAISFALYKAFSTNEHDRDNWNGQLKLLLEWNQLDLASDEIFTNDRNWESADLQDVMFTALVKDRPKFVRLFLENGLNLRKFLTTEVLRELYTNNFSSLVFKNLQIAKNSYNDALLTFVWKMVEDFRRGFKRYYKNSKDEMEIELSEECPITRHPLQALFIWSVLQNKKELSKVIWEQTRGCTLAALGASKLLKSMAKVKNDINAAGESEELANEYETRAVELFTECYSNDEDLAEQLLTYSCEAWGGSNCLELAVEARDQQFIAQPGVQNFLSKQWYGEISRDTKNWKIILCLFFFPLIGCGFISFRKKPVEKTKKLFLYYVSFFTSPFVVFSWNVIFYIAFLLLFAYVLLMDFQKEPTALEIILYVLVFILLCDEVRQWYMNGSKYFSDLWNVMDTLAIFYFIAGIVFRLHSDESSWYSGRVIFCLDYIVFTLRLIHIFTVSRNLGPKIIMLQRMMIDVFFFLFLFAVWMVAFGVARQGILRKNEHRWEWIFRSVIYEPYLAMFGQYPDDIDGTTYNFDHCTFSGNESKPLCVELDANNQPRFPEWITIPLVCIYMLSTNILLVNLLVAMFGYTVGSVQENNDQVWKFQRFFLVQEYCSRLTIPFPFVIFAYIFMVMRKCFKCCCKKESKEPSVCCSRNEDNEILAWEAVMKENYLVKINTKASDSSEDQTNTKNISLVLEAKVS

SEQ ID NO: 10 - protein, 839 aa, Homo sapiens [sequence omitted]

SEQ ID NO: 11 - protein, 730 aa, Oryctolagus cuniculus
MGACPPKAKGPWAQLQKLLISWPVGEQDWEQYRDRVNMLQQERIRDSPLLQAAKENDLRLLKILLLNQSCDFQQRGAVGETALHVAALYDNLEAATLLMEAAPELAKEPALCEPFVGQTALHIAVMNQNLNLVRALLARGASVSARATGAAFRRSPHNLIYYGEHPLSFAACVGSEEIVRLLIEHGADIRAQDSLGNTVLHILILQPNKTFACQMYNLLLSYDEHSDHLQSLELVPNHQGLTPFKLAGVEGNTVMFQHLMQKRKHVQWTCGPLTSTLYDLTEIDSWGEELSFLELVVSSKKREARQILEQTPVKELVSFKWKKYGRPYFCVLASLYILYMICFTTCCIYRPLKLRDDNRTDPRDITILQQKLLQEAYVTHQDNIRLVGELVTVTGAVIILLLEIPDIFRVGASRYFGQTILGGPFHVIIITYASLVLLTMVMRLTNMNGEVVPLSFALVLGWCSVMYFARGFQMLGPFTIMIQKMIFGDLMRFCWLMAVVILGFASAFHITFQTEDPNNLGEFSDYPTALFSTFELFLTIIDGPANYSVDLPFMYCITYAAFAIIATLLMLNLFIAMMGDTHWRVAQERDELWRAQVVATTVMLERKMPRFLWPRSGICGYEYGLGDRWFLRVENHHDQNPLRVLRYVEAFKCSDKEDGQEQLSEKRPSTVESGMLSRASVAFQTPSLSRTTSQSSNSHRGWEILRRNTLGHLNLGLDLGEGDGEEVYHF

SEQ ID NO: 12 - protein, 1119 aa, Homo sapiens
MKRSLRKMWRPGEKKEPQGVVYEDVPDDTEDFKESLKVVFEGSAYGLQNFNKQKKLKRCDDMDTFFLHYAAAEGQIELMEKITRDSSLEVLHEMDDYGNTPLHCAVEKNQIESVKFLLSRGANPNLRNFNMMAPLHIAVQGMNNEVMKVLLEHRTIDVNLEGENGNTAVIIACTTNNSEALQILLKKGAKPCKSNKWGCFPIHQAAFSGSKECMEIILRFGEEHGYSRQLHINFMNNGKATPLHLAVQNGDLEMIKMCLDNGAQIDPVEKGRCTAIHFAATQGATEIVKLMISSYSGSVDIVNTTDGCHETMLHRASLFDHHELADYLISVGADINKIDSEGRSPLILATASASWNIVNLLLSKGAQVDIKDNFGRNFLHLTVQQPYGLKNLRPEFMQMQQIKELVMDEDNDGCTPLHYACRQGGPGSVNNLLGFNVSIHSKSKDKKSPLHFAASYGRINTCQRLLQDISDTRLLNEGDLHGMTPLHLAAKNGHDKVVQLLLKKGALFLSDHNGWTALHHASMGGYTQTMKVILDTNLKCTDRLDEDGNTALHFAAREGHAKAVALLLSHNADIVLNKQQASFLHLALHNKRKEVVLTIIRSKRWDECLKIFSHNSPGNKCPITEMIEYLPECMKVLLDFCMLHSTEDKSCRDYYIEYNFKYLQCPLEFTKKTPTQDVIYEPLTALNAMVQNNRIELLNHPVCKEYLLMKWLAYGFRAHMMNLGSYCLGLIPMTILVVNIKPGMAFNSTGIINETSDHSEILDTTNSYLIKTCMILVFLSSIFGYCKEAGQIFQQKRNYFMDISNVLEWIIYTTGIIFVLPLFVEIPAHLQWQCGAIAVYFYWMNFLLYLQRFENCGIFIVMLEVILKTLLRSTVVFIFLLLAFGLSFYILLNLQDPFSSPLLSIIQTFSMMLGDINYRESFLEPYLRNELAHPVLSFAQLVSFTIFVPIVLMNLLIGLAVGDIAEVQKHASLKRIAMQVELHTSLEKKLPLWFLRKVDQKSTIVYPNKPRSGGMLFHIFCFLFCTGEIRQEIPNADKSLEMEILKQKYRLKDLTFLLEKQHELIKLIIQKMEIISETEDDDSHCSFQDRFKKEQMEQRNSRWNTVLRAVKAKTHHLEP

SEQ ID NO: 13 - protein, 1165 aa, synthetic construct
MVEKSSERFDKQMAGRLGDIDFTGVSRTRGKFVRVTSSTDPAEIYQILTKQWGLAPPHLVVALMGGDEVAQLKPWLRDTLRKGLVKAAQSTGAWILTSGLRFGITKNLGQAVRDHSLASTSPKVRVVAIGIAPWNMIQNRDLLLSAKPDHPATYPTEDLPYGAVYSLDCNHSHFILVDEDPKRPGATGEMRVKMLKHISLQRTGYGGTGSIEIPVLCLLVHGEPRILQKMYKNIQNSIPWLILAGSGGVADILVTLMDRGCWDADIVQELLINTFPDGLHSTEITSWTKLIQRILDHGHLLTVHDPEQDSELDTVILKALVKACKSQSQEAQDFLDELKLAVAWNRVDIAKSEIFSGDVQWSAQDLEEVMMEALVNDKPDFVRLFVDNGVNIKQFLTYGRLQELYCSVSEKNLLHTLLLKKNQERQAQLARKRMSGNPNNELGDRKFRFTFHEVSKVLKDFLDDTCKGFYQKLPAERMGKGRLFHSQKNLPDMDRRCEHPWRDLFLWAILQNRQEMANYFWAMGPEAVAAALVGCKIMKEMAHLATEAESARSMKNAKYEQFAMDLFSECYSNSEDRAYSLLVRKTCCWSKATVLNIATLAEAKCFFAHDGVQALLTKVWWGAMRTDTSISRLVLTFFIPPLVWTSLIKFNPEEQVSKDEGEPFAELDSLETEQALLLTDGDPVAGEGSAETAARSCSATFIRVVLRRWNRFWSAPVTVFMGNVIMYFAFLILFSYVLLLDFRPPPPYGPSAAEIILYFWVFTLVLEEIRQSFFTDEDMSILKKMKLYVEDNWNKCDMVAISLFVVGLSCRMAMSTYEAGRTVLALDFMVFTLRLIHIFAIHKQLGPKIIIVARMIKDVFFFLFFLSVWLIAYGVTTQALLHPNDPRIDWVFRRALYRPYLHIFGQIPLEEIDAAKMPDDNCTTDVQEIILGTLPPCPNIYANWLVILLLVIYLLVTNVLLLNLLIAMFSYTFQVVQENADIFWKFQRYNLIVEYHSRPALAPPFIIISHITQALLSFIKKTENTQDLLERELPSGLDQKLMTWETVQKENYLAKLEHEHRESSGERLRYTSSKVQTLLRMVGGFKDQEKRMATVETEVRYCGEVLSWIAECFHKSTLKCDRDAPKAPRSIAGSSRDQQPQGAKRQQPAGHPAYGTDKKLPFIDH

SEQ ID NO: 14 - protein, 1214 aa, synthetic construct
MVVPEKEQSWIPKIFKKKTCTTFIVDSTDPGGTLCQCGRPRTAHPAVAMEDAFGAAVVTVWDSDAHTTEKPTDAYGELDFTGAGRKHSNFLRLSDRTDPAAVYSLVTRTWGFRAPNLVVSVLGGSGGPVLQTWLQDLLRRGLVRAAQSTGAWIVTGGLHTGIGRHVGVAVRDHQMASTGGTKVVAMGVAPWGVVRNRDTLINPKGSFPARYRWRGDPEDGVQFPLDYNYSAFFLVDDGTHGCLGGENRFRLRLESYISQQKTGVGGTGIDIPVLLLLIDGDEKMLTRIENATQAQLPCLLVAGSGGAADCLAETLEDTLAPGSGGARQGEARDRIRRFFPKGDLEVLQAQVERIMTRKELLTVYSSEDGSEEFETIVLKALVKACGSSEASAYLDELRLAVAWNRVDIAQSELFRGDIQWRSFHLEASLMDALLNDRPEFVRLLISHGLSLGHFLTPMRLAQLYSAAPSNSLIRNLLDQASHSAGTKAPALKGGAAELRPPDVGHVLRMLLGKMCAPRYPSGGAWDPHPGQGFGESMYLLSDKATSPLSLDAGLGQAPWSDLLLWALLLNRAQMAMYFWEMGSNAVSSALGACLLLRVMARLEPDAEEAARRKDLAFKFEGMGVDLFGECYRSSEVRAARLLLRRCPLWGDATCLQLAMQADARAFFAQDGVQSLLTQKWWGDMASTTPIWALVLAFFCPPLIYTRLITFRKSEEEPTREELEFDMDSVINGEGPVGTADPAEKTPLGVPRQSGRPGCCGGRCGGRRCLRRWFHFWGAPVTIFMGNVVSYLLFLLLFSRVLLVDFQPAPPGSLELLLYFWAFTLLCEELRQGLSGGGGSLASGGPGPGHASLSQRLRLYLADSWNQCDLVALTCFLLGVGCRLTPGLYHLGRTVLCIDFMVFTVRLAHIFTVNKQLGPKIVIVAKMMKDVFFFLFFLGVWLVAYGVATEGLLRPRDSDFPSILRRVFYRPYLQIFGQIPQEDMDVALMEHSNCSSEPGFWAHPPGAQAGTCVSQYANWLVVLLLVIFLLVANILLVNLLIAMFSYTFGKVQGNSDLYWKAQRYRLIREFHSRPALAPPFIVISHLRLLLRQLCRRPRSPQPSSPALEHFRVYLSKEAERKLLTWESVHKENFLLARARDKRESDSERLKRTSQKVDLALKQLGHIREYEQRLKVLEREVQQCSRVLGWVAEALSRSALLPPGGPPPPDLPGSKD

SEQ ID NO: 15 - protein, 1165 aa, synthetic construct
MVEKSSERFDKQMAGRLGDIDFTGVSRTRGKFVRVTSSTDPAEIYQILTKQWGLAPPHLVVALMGGDEVAQLKPWLRDTLRKGLVKAAQSTGAWILTSGLRFGITKNLGQAVRDHSLASTSPKVRVVAIGIAPWNMIQNRDLLLSAKPDHPATYPTEDLPYGAVYSLDCNHSHFILVDEDPKRPGATGEMRVKMLKHISLQRTGYGGTGSIEIPVLCLLVHGEPRILQKMYKNIQNSIPWLILAGSGGVADILVTLMDRGCWDADIVQELLINTFPDGLHSTEITSWTKLIQRILDHGHLLTVHDPEQDSELDTVILKALVKACKSQSQEAQDFLDELKLAVAWNRVDIAKSEIFSGDVQWSAQDLEEVMMEALVNDKPDFVRLFVDNGVNIKQFLTYGRLQELYCSVSEKNLLHTLLLKKNQERQAQLARKRMSGNPNNELGDRKFRFTFHEVSKVLKDFLDDTCKGFYQKLPAERMGKGRLFHSQKNLPDMDRRCEHPWRDLFLWAILQNRQEMANYFWAMGPEAVAAALVGCKIMKEMAHLATEAESARSMKNAKYEQFAMDLFSECYSNSEDRAYSLLVRKTCCWSKATVLNIATLAEAKCFFAHDGVQALLTKVWWGAMRTDTSISRLVLTFFIPPLVWTSLIKFNPEEQVSKDEGEPFAELDSLETEQALLLTDGDPVAGEGSAETAARSCSATFIRVVLRRWNRFWSAPVTVFMGNVIMYFAFLILFSYVLLLDFRPPPPYGPSAAEIILYFWVFTLVLEEIRQSFFTDEDMSILKKMKLYVEDNWNKCDMVAISLFVVGLSCRMAMSTYEAGRTVLALDFMVFTLRLAHIFAIHKQLGPKIIIVERMIKDVFFFLFFLSVWLIAYGVTTQALLHPNDPRIDWVFRRALYRPYLHIFGQIPLEEIDAAKMPDDNCTTDVQEIILGTLPPCPNIYANWLVILLLVIYLLVTNVLLLNLLIAMFSYTFQVVQENADIFWKFQRYNLIVEYHSRPALAPPFIIISHITQALLSFIKKTENTQDLLERELPSGLDQKLMTWETVQKENYLAKLEHEHRESSGERLRYTSSKVQTLLRMVGGFKDQEKRMATVETEVRYCGEVLSWIAECFHKSTLKCDRDAPKAPRSIAGSSRDQQPQGAKRQQPAGHPAYGTDKKLPFIDH

SEQ ID NO: 16 - protein, 1165 aa, synthetic construct
MVEKSSERFDKQMAGRLGDIDFTGVSRTRGKFVRVTSSTDPAEIYQILTKQWGLAPPHLVVALMGGDEVAQLKPWLRDTLRKGLVKAAQSTGAWILTSGLRFGITKNLGQAVRDHSLASTSPKVRVVAIGIAPWNMIQNRDLLLSAKPDHPATYPTEDLPYGAVYSLDCNHSHFILVDEDPKRPGATGEMRVKMLKHISLQRTGYGGTGSIEIPVLCLLVHGEPRILQKMYKNIQNSIPWLILAGSGGVADILVTLMDRGCWDADIVQELLINTFPDGLHSTEITSWTKLIQRILDHGHLLTVHDPEQDSELDTVILKALVKACKSQSQEAQDFLDELKLAVAWNRVDIAKSEIFSGDVQWSAQDLEEVMMEALVNDKPDFVRLFVDNGVNIKQFLTYGRLQELYCSVSEKNLLHTLLLKKNQERQAQLARKRMSGNPNNELGDRKFRFTFHEVSKVLKDFLDDTCKGFYQKLPAERMGKGRLFHSQKNLPDMDRRCEHPWRDLFLWAILQNRQEMANYFWAMGPEAVAAALVGCKIMKEMAHLATEAESARSMKNAKYEQFAMDLFSECYSNSEDRAYSLLVRKTCCWSKATVLNIATLAEAKCFFAHDGVQALLTKVWWGAMRTDTSISRLVLTFFIPPLVWTSLIKFNPEEQVSKDEGEPFAELDSLETEQALLLTDGDPVAGEGSAETAARSCSATFIRVVLRRWNRFWSAPVTVFMGNVIMYFAFLILFSYVLLLDFRPPPPYGPSAAEIILYFWVFTLVLEEIRQSFFTDEDMSILKKMKLYVEDNWNKCDMVAISLFVVGLSCRMAMSTYEAGRTVLALDFMVFTARLIHIFAIHKQLGPKIIIVERMIKDVFFFLFFLSVWLIAYGVTTQALLHPNDPRIDWVFRRALYRPYLHIFGQIPLEEIDAAKMPDDNCTTDVQEIILGTLPPCPNIYANWLVILLLVIYLLVTNVLLLNLLIAMFSYTFQVVQENADIFWKFQRYNLIVEYHSRPALAPPFIIISHITQALLSFIKKTENTQDLLERELPSGLDQKLMTWETVQKENYLAKLEHEHRESSGERLRYTSSKVQTLLRMVGGFKDQEKRMATVETEVRYCGEVLSWIAECFHKSTLKCDRDAPKAPRSIAGSSRDQQPQGAKRQQPAGHPAYGTDKKLPFIDH

SEQ ID NO: 17 - protein, 1165 aa, synthetic construct
MVEKSSERFDKQMAGRLGDIDFTGVSRTRGKFVRVTSSTDPAEIYQILTKQWGLAPPHLVVALMGGDEVAQLKPWLRDTLRKGLVKAAQSTGAWILTSGLRFGITKNLGQAVRDHSLASTSPKVRVVAIGIAPWNMIQNRDLLLSAKPDHPATYPTEDLPYGAVYSLDCNHSHFILVDEDPKRPGATGEMRVKMLKHISLQRTGYGGTGSIEIPVLCLLVHGEPRILQKMYKNIQNSIPWLILAGSGGVADILVTLMDRGCWDADIVQELLINTFPDGLHSTEITSWTKLIQRILDHGHLLTVHDPEQDSELDTVILKALVKACKSQSQEAQDFLDELKLAVAWNRVDIAKSEIFSGDVQWSAQDLEEVMMEALVNDKPDFVRLFVDNGVNIKQFLTYGRLQELYCSVSEKNLLHTLLLKKNQERQAQLARKRMSGNPNNELGDRKFRFTFHEVSKVLKDFLDDTCKGFYQKLPAERMGKGRLFHSQKNLPDMDRRCEHPWRDLFLWAILQNRQEMANYFWAMGPEAVAAALVGCKIMKEMAHLATEAESARSMKNAKYEQFAMDLFSECYSNSEDRAYSLLVRKTCCWSKATVLNIATLAEAKCFFAHDGVQALLTKVWWGAMRTDTSISRLVLTFFIPPLVWTSLIKFNPEEQVSKDEGEPFAELDSLETEQALLLTDGDPVAGEGSAETAARSCSATFIRVVLRRWNRFWSAPVTVFMGNVIMYFAFLILFSYVLLLDFRPPPPYGPSAAEIILYFWVFTLVLEEIRQSFFTDEDMSILKKMKLYVEDNWNKCDMVAISLFVVGLSCRMAMSTYEAGRTVLALDFMVFTLRLIHIFAIHKQLGPKIIIVERMIKDVFFFLFFLSVALIAYGVTTQALLHPNDPRIDWVFRRALYRPYLHIFGQIPLEEIDAAKMPDDNCTTDVQEIILGTLPPCPNIYANWLVILLLVIYLLVTNVLLLNLLIAMFSYTFQVVQENADIFWKFQRYNLIVEYHSRPALAPPFIIISHITQALLSFIKKTENTQDLLERELPSGLDQKLMTWETVQKENYLAKLEHEHRESSGERLRYTSSKVQTLLRMVGGFKDQEKRMATVETEVRYCGEVLSWIAECFHKSTLKCDRDAPKAPRSIAGSSRDQQPQGAKRQQPAGHPAYGTDKKLPFIDH